European Patent Specification EP 3 652 214 B1, published February 25, 2026. Title: New binding agent and assay for PIVKA. Applicant: Roche Diagnostics GmbH F. Hoffmann-La Roche AG. The sequence listing filed with the application follows.

SEQUENCE LISTING (34 sequences)

SEQ ID NO: 1 - protein, 16 aa, Artificial Sequence
  synthetic peptide
NLERECVEETCSYEEA

SEQ ID NO: 2 - protein, 16 aa, Artificial sequence
  synthetic peptide
  Xaa (8)..(8): Xaa is gamma-carboxylated glutamic acid
NLERECVXETCSYEEA

SEQ ID NO: 3 - protein, 16 aa, Artificial sequence
  synthetic peptide
  Xaa (13)..(13): Xaa represents gamma carboxylated glutamic acid
  misc_feature (14)..(14): Xaa can be any naturally occurring amino acid
NLERECVEETCSYXEA

SEQ ID NO: 4 - protein, 16 aa, Artificial sequence
  synthetic peptide
  Xaa (9)..(9): Xaa represents gamma carboxylated glutamic acid
NLERECVEXTCSYEEA

SEQ ID NO: 5 - protein, 622 aa, Homo sapiens
MAHVRGLQLPGCLALAALCSLVHSQHVFLAPQQARSLLQRVRRANTFLEEVRKGNLERECVEETCSYEEAFEALESSTATDVFWAKYTACETARTPRDKLAACLEGNCAEGLGTNYRGHVNITRSGIECQLWRSRYPHKPEINSTTHPGADLQENFCRNPDSSTTGPWCYTTDPTVRRQECSIPVCGQDQVTVAMTPRSEGSSVNLSPPLEQCVPDRGQQYQGRLAVTTHGLPCLAWASAQAKALSKHQDFNSAVQLVENFCRNPDGDEEGVWCYVAGKPGDFGYCDLNYCEEAVEEETGDGLDEDSDRAIEGRTATSEYQTFFNPRTFGSGEADCGLRPLFEKKSLEDKTERELLESYIDGRIVEGSDAEIGMSPWQVMLFRKSPQELLCGASLISDRWVLTAAHCLLYPPWDKNFTENDLLVRIGKHSRTRYERNIEKISMLEKIYIHPRYNWRENLDRDIALMKLKKPVAFSDYIHPVCLPDRETAASLLQAGYKGRVTGWGNLKETWTANVGKGQPSVLQVVNLPIVERPVCKDSTRIRITDNMFCAGYKPDEGKRGDACEGDSGGPFVMKSPFNNRWYQMGIVSWGEGCDRDGKYGFYTHVFRLKKWIQKVIDQFGE

SEQ ID NO: 6 - protein, 579 aa, Homo sapiens
ANTFLEEVRKGNLERECVEETCSYEEAFEALESSTATDVFWAKYTACETARTPRDKLAACLEGNCAEGLGTNYRGHVNITRSGIECQLWRSRYPHKPEINSTTHPGADLQENFCRNPDSSTTGPWCYTTDPTVRRQECSIPVCGQDQVTVAMTPRSEGSSVNLSPPLEQCVPDRGQQYQGRLAVTTHGLPCLAWASAQAKALSKHQDFNSAVQLVENFCRNPDGDEEGVWCYVAGKPGDFGYCDLNYCEEAVEEETGDGLDEDSDRAIEGRTATSEYQTFFNPRTFGSGEADCGLRPLFEKKSLEDKTERELLESYIDGRIVEGSDAEIGMSPWQVMLFRKSPQELLCGASLISDRWVLTAAHCLLYPPWDKNFTENDLLVRIGKHSRTRYERNIEKISMLEKIYIHPRYNWRENLDRDIALMKLKKPVAFSDYIHPVCLPDRETAASLLQAGYKGRVTGWGNLKETWTANVGKGQPSVLQVVNLPIVERPVCKDSTRIRITDNMFCAGYKPDEGKRGDACEGDSGGPFVMKSPFNNRWYQMGIVSWGEGCDRDGKYGFYTHVFRLKKWIQKVIDQFGE

SEQ ID NO: 7 - protein, 46 aa, Homo sapiens
ANTFLEEVRKGNLERECVEETCSYEEAFEALESSTATDVFWAKYTA

SEQ ID NO: 8 - protein, 225 aa, Homo sapiens
CETARTPRDKLAACLEGNCAEGLGTNYRGHVNITRSGIECQLWRSRYPHKPEINSTTHPGADLQENFCRNPDSSTTGPWCYTTDPTVRRQECSIPVCGQDQVTVAMTPRSEGSSVNLSPPLEQCVPDRGQQYQGRLAVTTHGLPCLAWASAQAKALSKHQDFNSAVQLVENFCRNPDGDEEGVWCYVAGKPGDFGYCDLNYCEEAVEEETGDGLDEDSDRAIEGR

SEQ ID NO: 9 - protein, 155 aa, Homo sapiens
ANTFLEEVRKGNLERECVEETCSYEEAFEALESSTATDVFWAKYTACETARTPRDKLAACLEGNCAEGLGTNYRGHVNITRSGIECQLWRSRYPHKPEINSTTHPGADLQENFCRNPDSSTTGPWCYTTDPTVRRQECSIPVCGQDQVTVAMTPR

SEQ ID NO: 10 - protein, 11 aa, Mus musculus
QASQSIGNNLA

SEQ ID NO: 11 - protein, 7 aa, Mus musculus
SASTLAS

SEQ ID NO: 12 - protein, 14 aa, Mus musculus
QSYAGVSESVFWYS

SEQ ID NO: 13 - protein, 13 aa, Mus musculus
TVSGIDLSTYAMG

SEQ ID NO: 14 - protein, 16 aa, Mus musculus
IIRSSGRTYYASWAKG

SEQ ID NO: 15 - protein, 4 aa, Mus musculus
NVSL

SEQ ID NO: 16 - protein, 112 aa, Mus musculus
DVVMTQTPSSVEAAVGGTVTIKCQASQSIGNNLAWYQQKPGQRPNLLIYSASTLASGVPSRFRGSGSGTEFTLTISGVQCDDAATYYCQSYAGVSESVFWYSFGGGTGVVVK

SEQ ID NO: 17 - protein, 110 aa, Mus musculus
QSLEESGGRLVTPGTPLTLTCTVSGIDLSTYAMGWVRQAPGKGLEYIGIIRSSGRTYYASWAKGRFTVSKTSSTTVDLSMTSPTTEDTATYYCYRNVSLWGQGTLVSVSS

SEQ ID NO: 18 - protein, 11 aa, Mus musculus
QASQSIGSNLA

SEQ ID NO: 19 - protein, 7 aa, Mus musculus
SASTLAP

SEQ ID NO: 20 - protein, 14 aa, Mus musculus
QSYAGVSANIFYYS

SEQ ID NO: 21 - protein, 13 aa, Mus musculus
TVSGFDLSRYAVG

SEQ ID NO: 22 - protein, 16 aa, Mus musculus
LITSDGRTYYANWAKG

SEQ ID NO: 23 - protein, 112 aa, Mus musculus
DVVMTQTPASVEAAVGGTVTIKCQASQSIGSNLAWYQQKSGQPPKLLIYSASTLAPGVSSRFSGSGSGTEFTLTFTGVQCGDAATYFCQSYAGVSANIFYYSFGGGTEVVVM

SEQ ID NO: 24 - protein, 110 aa, Mus musculus
QSVEESGGRLVTPGTPLTLTCTVSGFDLSRYAVGWVRQAPGKGLEYIGLITSDGRTYYANWAKGRFTVSKTSSTTVDLKMTSPTTEDTATYYCYRNVSLWGQGTLVSVSS

SEQ ID NO: 25 - protein, 16 aa, Mus musculus
LIVSDGRTYYASWAKG

SEQ ID NO: 26 - protein, 112 aa, Mus musculus
DVVMTQTPSSVEAAVGGTVTIKCQASQSIGSNLAWYQQKPGQPPKLLIYSASTLASGVPSRFSGSGSGTEFTLTFSGVQCGDAATYFCQSYAGVSANIFYYSFGGGTEVVVM

SEQ ID NO: 27 - protein, 110 aa, Mus musculus
QSVEESGGRLITPGTPLTLTCTVSGFDLSRYAVGWVRQAPGKGLEYIGLIVSDGRTYYASWAKGRFTVSKTSSTTVDLKMTSPTAGDTATYYCYRNVSLWGQGTLVSVSS

SEQ ID NO: 28 - protein, 14 aa, Mus musculus
QSYAGISANIFYYA

SEQ ID NO: 29 - protein, 13 aa, Mus musculus
TVSGFDLSRYAMG

SEQ ID NO: 30 - protein, 112 aa, Mus musculus
DVVMTQTPSSVEAAVGGTVTIKCQASQSIGSNLAWYQQKPGQPPKLLIYSASTLASGVSSRFKGSGSGTEFTLTISDLECADAATYYCQSYAGISANIFYYAFGGGTEVVVM

SEQ ID NO: 31 - protein, 110 aa, Mus musculus
QSVEESGGRLVTPETPLTLTCTVSGFDLSRYAMGWVRQAPGKGLEYIGLIVSDGRTYYASWAKGRFTISKTSSTTVDLKMASPTTEDTATYYCYRNVSLWGQGTLVSVSE

SEQ ID NO: 32 - protein, 27 aa, artificial sequence
  synthetic peptide
  Xaa (1)..(4): Xaa in positions 1, 3 and 4 is beta alanine; Xaa in position 2 is 6-aminohexanoic acid
XXXXVRRGNLERECVEETCSYEEAFEA

SEQ ID NO: 33 - protein, 20 aa, artificial sequence
  synthetic peptide
  Xaa (1)..(4): Xaa in positions 1, 3 and 4 is beta alanine; Xaa in position 2 is 6-aminohexanoic acid
XXXXNLERECVEETCSYEEA

SEQ ID NO: 34 - protein, 20 aa, artificial sequence
  synthetic peptide
  Xaa (17)..(19): Xaa in positions 17 and 19 is beta alanine; Xaa in position 18 is 6-aminohexanoic acid
ANTFLEEVRKGNLEREXXXC